European Patent Application EP 4 249 588 A1, published September 27, 2023. Title: CELLULAR THERAPY. Applicant: Hornet Therapeutics Limited. The sequence listing filed with the application follows.

SEQUENCE LISTING (4 sequences)

SEQ ID NO: 1 - protein, 533 aa, Homo sapiens
MAFANLRKVLISDSLDPCCRKILQDGGLQVVEKQNLSKEELIAELQDCEGLIVRSATKVTADVINAAEKLQVVGRAGTGVDNVDLEAATRKGILVMNTPNGNSLSAAELTCGMIMCLARQIPQATASMKDGKWERKKFMGTELNGKTLGILGLGRIGREVATRMQSFGMKTIGYDPIISPEVSASFGVQQLPLEEIWPLCDFITVHTPLLPSTTGLLNDNTFAQCKKGVRVVNCARGGIVDEGALLRALQSGQCAGAALDVFTEEPPRDRALVDHENVISCPHLGASTKEAQSRCGEEIAVQFVDMVKGKSLTGVVNAQALTSAFSPHTKPWIGLAEALGTLMRAWAGSPKGTIQVITQGTSLKNAGNCLSPAVIVGLLKEASKQADVNLVNAKLLVKEAGLNVTTSHSPAAPGEQGFGECLLAVALAGAPYQAVGLVQGTTPVLQGLNGAVFRPEVPLRRDLPLLLFRTQTSDPAMLPTMIGLLAEAGVRLLSYQTSLVSDGETWHVMGISSLLPSLEAWKQHVTEAFQFHF

SEQ ID NO: 2 - DNA, 1617 bp, Homo sapiens
atgaagcttatggcttttgcaaatctgcggaaagtgctcatcagtgacagcctggacccttgctgccggaagatcttgcaagatggagggctgcaggtggtggaaaagcagaaccttagcaaagaggagctgatagcggagctgcaggactgtgaaggccttattgttcgctctgccaccaaggtgaccgctgatgtcatcaacgcagctgagaaactccaggtggtgggcagggctggcacaggtgtggacaatgtggatctggaggccgcaacaaggaagggcatcttggttatgaacacccccaatgggaacagcctcagtgccgcagaactcacttgtggaatgatcatgtgcctggccaggcagattccccaggcgacggcttcgatgaaggacggcaaatgggagcggaagaagttcatgggaacagagctgaatggaaagaccctgggaattcttggcctgggcaggattgggagagaggtagctacccggatgcagtcctttgggatgaagactatagggtatgaccccatcatttccccagaggtctcggcctcctttggtgttcagcagctgcccctggaggagatctggcctctctgtgatttcatcactgtgcacactcctctcctgccctccacgacaggcttgctgaatgacaacacctttgcccagtgcaagaagggggtgcgtgtggtgaactgtgcccgtggagggatcgtggacgaaggcgccctgctccgggccctgcagtctggccagtgtgccggggctgcactggacgtgtttacggaagagccgccacgggaccgggccttggtggaccatgagaatgtcatcagctgtccccacctgggtgccagcaccaaggaggctcagagccgctgtggggaggaaattgctgttcagttcgtggacatggtgaaggggaaatctctcacgggggttgtgaatgcccaggcccttaccagtgccttctctccacacaccaagccttggattggtctggcagaagctctggggacactgatgcgagcctgggctgggtcccccaaagggaccatccaggtgataacacagggaacatccctgaagaatgctgggaactgcctaagccccgcagtcattgtcggcctcctgaaagaggcttccaagcaggcggatgtgaacttggtgaacgctaagctgctggtgaaagaggctggcctcaatgtcaccacctcccacagccctgctgcaccaggggagcaaggcttcggggaatgcctcctggccgtggccctggcaggcgccccttaccaggctgtgggcttggtccaaggcactacgcctgtactgcaggggctcaatggagctgtcttcaggccagaagtgcctctccgcagggacctgcccctgctcctattccggactcagacctctgaccctgcaatgctgcctaccatgattggcctcctggcagaggcaggcgtgcggctgctgtcctaccagacttcactggtgtcagatggggagacctggcacgtcatgggcatctcctccttgctgcccagcctggaagcgtggaagcagcatgtgactgaagccttccagttccacttctaaggatcc

SEQ ID NO: 3 - protein, 533 aa, Artificial Sequence
  Phosphoglycerate dehydrogenase (catalytically dead), R236E
MAFANLRKVLISDSLDPCCRKILQDGGLQVVEKQNLSKEELIAELQDCEGLIVRSATKVTADVINAAEKLQVVGRAGTGVDNVDLEAATRKGILVMNTPNGNSLSAAELTCGMIMCLARQIPQATASMKDGKWERKKFMGTELNGKTLGILGLGRIGREVATRMQSFGMKTIGYDPIISPEVSASFGVQQLPLEEIWPLCDFITVHTPLLPSTTGLLNDNTFAQCKKGVRVVNCAEGGIVDEGALLRALQSGQCAGAALDVFTEEPPRDRALVDHENVISCPHLGASTKEAQSRCGEEIAVQFVDMVKGKSLTGVVNAQALTSAFSPHTKPWIGLAEALGTLMRAWAGSPKGTIQVITQGTSLKNAGNCLSPAVIVGLLKEASKQADVNLVNAKLLVKEAGLNVTTSHSPAAPGEQGFGECLLAVALAGAPYQAVGLVQGTTPVLQGLNGAVFRPEVPLRRDLPLLLFRTQTSDPAMLPTMIGLLAEAGVRLLSYQTSLVSDGETWHVMGISSLLPSLEAWKQHVTEAFQFHF

SEQ ID NO: 4 - DNA, 1617 bp, Artificial Sequence
  Encodes phosphoglycerate dehydrogenase (catalytically dead), R236E
atgaagcttatggcttttgcaaatctgcggaaagtgctcatcagtgacagcctggacccttgctgccggaagatcttgcaagatggagggctgcaggtggtggaaaagcagaaccttagcaaagaggagctgatagcggagctgcaggactgtgaaggccttattgttcgctctgccaccaaggtgaccgctgatgtcatcaacgcagctgagaaactccaggtggtgggcagggctggcacaggtgtggacaatgtggatctggaggccgcaacaaggaagggcatcttggttatgaacacccccaatgggaacagcctcagtgccgcagaactcacttgtggaatgatcatgtgcctggccaggcagattccccaggcgacggcttcgatgaaggacggcaaatgggagcggaagaagttcatgggaacagagctgaatggaaagaccctgggaattcttggcctgggcaggattgggagagaggtagctacccggatgcagtcctttgggatgaagactatagggtatgaccccatcatttccccagaggtctcggcctcctttggtgttcagcagctgcccctggaggagatctggcctctctgtgatttcatcactgtgcacactcctctcctgccctccacgacaggcttgctgaatgacaacacctttgcccagtgcaagaagggggtgcgtgtggtgaactgtgccgagggagggatcgtggacgaaggcgccctgctccgggccctgcagtctggccagtgtgccggggctgcactggacgtgtttacggaagagccgccacgggaccgggccttggtggaccatgagaatgtcatcagctgtccccacctgggtgccagcaccaaggaggctcagagccgctgtggggaggaaattgctgttcagttcgtggacatggtgaaggggaaatctctcacgggggttgtgaatgcccaggcccttaccagtgccttctctccacacaccaagccttggattggtctggcagaagctctggggacactgatgcgagcctgggctgggtcccccaaagggaccatccaggtgataacacagggaacatccctgaagaatgctgggaactgcctaagccccgcagtcattgtcggcctcctgaaagaggcttccaagcaggcggatgtgaacttggtgaacgctaagctgctggtgaaagaggctggcctcaatgtcaccacctcccacagccctgctgcaccaggggagcaaggcttcggggaatgcctcctggccgtggccctggcaggcgccccttaccaggctgtgggcttggtccaaggcactacgcctgtactgcaggggctcaatggagctgtcttcaggccagaagtgcctctccgcagggacctgcccctgctcctattccggactcagacctctgaccctgcaatgctgcctaccatgattggcctcctggcagaggcaggcgtgcggctgctgtcctaccagacttcactggtgtcagatggggagacctggcacgtcatgggcatctcctccttgctgcccagcctggaagcgtggaagcagcatgtgactgaagccttccagttccacttctaaggatcc